European Patent Application EP 4 144 865 A1, published March 8, 2023. Title: Microparticle probe for nucleic acid separation and detection for multiplexed diagnosis. Applicant: EZdiatech. The sequence listing filed with the application follows.

SEQUENCE LISTING (16 sequences)

SEQ ID NO: 1 - RNA, 288 nt, Artificial Sequence
  Covid 19
gggcgaauuggguaccaacacaagcuuucggcagacgugguccagaacaaacccaaggaaauuuuggggaccaggaacuaaucagacaaggaacugauuacaaacauuggccgcaaauugcacaauuugcccccagcgcuucagcguucuucggaaugucgcgcauuggcauggaagucacaccuucgggaacgugguugaccuacacaggugccaucaaauuggaugacaaagauccaaauuucaagcuugauaucgaauuccugcagcccgggggauccacuaguu

SEQ ID NO: 2 - DNA, 288 bp, Artificial Sequence
  Covid 19
gggcgaauuggguaccaacacaagcuuucggcagacgugguccagaacaaacccaaggaaauuuuggggaccaggaacuaaucagacaaggaacugauuacaaacauuggccgcaaauugcacaauuugcccccagcgcuucagcguucuucggaaugucgcgcauuggcauggaagucacaccuucgggaacgugguugaccuacacaggugccaucaaauuggaugacaaagauccaaauuucaagcuugauaucgaauuccugcagcccgggggauccacuaguu

SEQ ID NO: 3 - DNA, 229 bp, Artificial Sequence
  Covid 19
aacacaagctttcggcagacgtggtccagaacaaacccaaggaaattttggggaccaggaactaatcagacaaggaactgattacaaacattggccgcaaattgcacaatttgcccccagcgcttcagcgttcttcggaatgtcgcgcattggcatggaagtcacaccttcgggaacgtggttgacctacacaggtgccatcaaattggatgacaaagatccaaatttc

SEQ ID NO: 4 - DNA, 181 bp, Artificial Sequence
  Covid 19
ccgggagacaaaataacattcgaagcaactggaaatctagtggtaccgagatatgcattcgcaatggaaagaaatgctggatctggtattatcatttcagatacaccagtccacgattgcaatacaacttgtcagacacccaagggtgctataaacaccagcctcccatttcagaatatac

SEQ ID NO: 5 - DNA, 153 bp, Artificial Sequence
  Covid 19
atgtcgctgtttggagacacaattgcctacctgctttcattgacagaagatggagaaggcaaagcagaactagcagaaaaattacactgttggttcggtgggaaagaatttgacctagactctgctttggaatggataaaaaacaaaagatgc

SEQ ID NO: 6 - DNA, 18 bp, Artificial Sequence
  Forward Primer of RPA
aacacaagctttcggcag

SEQ ID NO: 7 - DNA, 22 bp, Artificial Sequence
  Reverse Primer of RPA
gaaatttggatctttgtcatcc

SEQ ID NO: 8 - DNA, 21 bp, Artificial Sequence
  Forward Primer of RPA
ccgggagacaaaataacattc

SEQ ID NO: 9 - DNA, 21 bp, Artificial Sequence
  Reverse Primer of RPA
gtatattctgaaatgggaggc

SEQ ID NO: 10 - DNA, 25 bp, Artificial Sequence
  Forward Primer of RPA
atgtcgctgtttggagacacaattg

SEQ ID NO: 11 - DNA, 24 bp, Artificial Sequence
  gRNA
gcatcttttgttttttatccattc

SEQ ID NO: 12 - RNA, 41 nt, Artificial Sequence
  gRNA targeting Covid 19
uaauuucuacuaaguguagaucccccagcgcuucagcguuc

SEQ ID NO: 13 - RNA, 41 nt, Artificial Sequence
  gRNA targeting Influenza A
uaauuucuacuaaguguagauagauacaccaguccacgauu

SEQ ID NO: 14 - RNA, 41 nt, Artificial Sequence
  gRNA targeting Influenza B
uaauuucuacuaaguguagauauugacagaagauggagaag

SEQ ID NO: 15 - DNA, 8 bp, Artificial Sequence
  Reporter DNA
ttattatt

SEQ ID NO: 16 - DNA, 10 bp, Artificial Sequence
  Reporter DNA
ttattatttt